European Patent Application EP 4 467 648 A2, published November 27, 2024. Title: ANTI-DR5 ANTIBODIES AND METHODS OF USE THEREOF. Applicant: Genmab B.V. Application EP PCT/EP2016/079518, filed December 1, 2016. The sequence listing filed with the application follows.

SEQUENCE LISTING (68 sequences)

SEQ ID NO: 1 - protein, 8 aa, synthetic construct
  REGION 1..8: note = N/A
GFNIKDTF

SEQ ID NO: 2 - protein, 8 aa, synthetic construct
  REGION 1..8: note = N/A
IDPANGNT

SEQ ID NO: 3 - protein, 11 aa, synthetic construct
  REGION 1..11: note = N/A
VRGLYTYYFDY

SEQ ID NO: 4 - protein, 118 aa, synthetic construct
  REGION 1..118: note = N/A
EVQLQQSGAEVVKPGASVKLSCKASGFNIKDTFIHWVKQAPGQGLEWIGRIDPANGNTKYDPKFQGKATITTDTSSNTAYMELSSLRSEDTAVYYCVRGLYTYYFDYWGQGTLVTVSS

SEQ ID NO: 5 - protein, 6 aa, synthetic construct
  REGION 1..6: note = N/A
QSISNN

SEQ ID NO: 6 - protein, 9 aa, synthetic construct
  REGION 1..9: note = N/A
QQGNSWPYT

SEQ ID NO: 7 - protein, 107 aa, synthetic construct
  REGION 1..107: note = N/A
EIVMTQSPATLSVSPGERATLSCRASQSISNNLHWYQQKPGQAPRLLIKFASQSITGIPARFSGSGSGTEFTLTISSLQSEDFAVYYCQQGNSWPYTFGQGTKLEIK

SEQ ID NO: 8 - protein, 8 aa, synthetic construct
  REGION 1..8: note = N/A
IDPANTNT

SEQ ID NO: 9 - protein, 118 aa, synthetic construct
  REGION 1..118: note = N/A
EVQLQQSGAEVVKPGASVKLSCKASGFNIKDTFIHWVKQAPGQGLEWIGRIDPANTNTKYDPKFQGKATITTDTSSNTAYMELSSLRSEDTAVYYCVRGLYTYYFDYWGQGTLVTVSS

SEQ ID NO: 10 - protein, 8 aa, synthetic construct
  REGION 1..8: note = N/A
GFNIKDTH

SEQ ID NO: 11 - protein, 11 aa, synthetic construct
  REGION 1..11: note = N/A
ARWGTNVYFAY

SEQ ID NO: 12 - protein, 118 aa, synthetic construct
  REGION 1..118: note = N/A
QVQLVQSGAEVKKPGASVKVSCKASGFNIKDTHMHWVRQAPGQRLEWIGRIDPANGNTEYDQKFQGRVTITVDTSASTAYMELSSLRSEDTAVYYCARWGTNVYFAYWGQGTLVTVSS

SEQ ID NO: 13 - protein, 5 aa, synthetic construct
  REGION 1..5: note = N/A
SSVSY

SEQ ID NO: 14 - protein, 9 aa, synthetic construct
  REGION 1..9: note = N/A
QQYHSYPPT

SEQ ID NO: 15 - protein, 106 aa, synthetic construct
  REGION 1..106: note = N/A
DIQLTQSPSSLSASVGDRVTITCSASSSVSYMYWYQQKPGKAPKPWIYRTSNLASGVPSRFSGSGSGTDFTLTISSLQPEDFATYYCQQYHSYPPTFGGGTKVEIK

SEQ ID NO: 16 - protein, 10 aa, synthetic construct
  REGION 1..10: note = N/A
GGSISSGDYF

SEQ ID NO: 17 - protein, 7 aa, synthetic construct
  REGION 1..7: note = N/A
IHNSGTT

SEQ ID NO: 18 - protein, 14 aa, synthetic construct
  REGION 1..14: note = N/A
ARDRGGDYYYGMDV

SEQ ID NO: 19 - protein, 122 aa, synthetic construct
  REGION 1..122: note = N/A
QVQLQESGPGLVKPSQTLSLTCTVSGGSISSGDYFWSWIRQLPGKGLECIGHIHNSGTTYYNPSLKSRVTISVDTSKKQFSLRLSSVTAADTAVYYCARDRGGDYYYGMDVWGQGTTVTVSS

SEQ ID NO: 20 - protein, 122 aa, synthetic construct
  REGION 1..122: note = N/A
QVQLQESGPGLVKPSQTLSLTCTVSGGSISSGDYFWSWIRQLPGKGLEWIGHIHNSGTTYYNPSLKSRVTISVDTSKKQFSLRLSSVTAADTAVYYCARDRGGDYYYGMDVWGQGTTVTVSS

SEQ ID NO: 21 - protein, 7 aa, synthetic construct
  REGION 1..7: note = N/A
QGISRSY

SEQ ID NO: 22 - protein, 9 aa, synthetic construct
  REGION 1..9: note = N/A
QQFGSSPWT

SEQ ID NO: 23 - protein, 108 aa, synthetic construct
  REGION 1..108: note = N/A
EIVLTQSPGTLSLSPGERATLSCRASQGISRSYLAWYQQKPGQAPSLLIYGASSRATGIPDRFSGSGSGTDFTLTISRLEPEDFAVYYCQQFGSSPWTFGQGTKVEIK

SEQ ID NO: 24 - protein, 439 aa, Homo sapiens
MEQRGQNAPAASGARKRHGPGPREARGARPGPRVPKTLVLVVAAVLLLVSAESALITQQDLAPQQRAAPQQKRSSPSEGLCPPGHHISEDGRDCISCKYGQDYSTHWNDLLFCLRCTRCDSGEVELSPCTTTRNTVCQCEEGTFREEDSPEMCRKCRTGCPRGMVKVGDCTPWSDIECVHKESGTKHSGEVPAVEETVTSSPGTPASPCSLSGIIIGVTVAAVVLIVAVFVCKSLLWKKVLPYLKGICSGGGGDPERVDRSSQRPGAEDNVLNEIVSILQPTQVPEQEMEVQEPAEPTGVNMLSPGESEHLLEPAEAERSQRRRLLVPANEGDPTETLRQCFDDFADLVPFDSWEPLMRKLGLMDNEIKVAKAEAAGHRDTLYTMLIKWVNKTGRDASVHTLLDALETLGERLAKKIEDHLLSSGKFMYLEGNADSAMS

SEQ ID NO: 25 - protein, 440 aa, Macaca mulatta
MGQLRQSAPAASGARKGRGPGPREARGARPGLRVLKTLVLVVAAARVLVSADCAPITRQSLDPQRRAAPQQKRSSPTEGLCPPGHHISEDSRDCISCKYGQDYSTHWNDFLFCLRCTKCDSGEVEVNSCTTTRNTVCQCEEGTFREEDSPEICRKCRTGCPRGMVKVKDCTPWSDIECVHKESGTKHTGEVPAVEKTVTTSPGTPASPCSLSGIIIGVIVFVVIVVVAVIVWKTSLWKKVLPYLKGVCSGDGGDPERVDSSPQRPGAEDNALNEIVSIVQPSQVPEQEMEVQEPAEQTDVNTLSPGESEHLLEPAKAEGPQRRGQLVPVNENDPTETLRQCFDDFAAIVPFDAWEPLVRQLGLTNNEIKVAKAEAASSRDTLYVMLIKWVNKTGRAASVNTLLDALETLEERLAKQKIQDRLLSSGKFMYLEDNADSATS

SEQ ID NO: 26 - protein, 381 aa, Mus musculus
MEPPGPSTPTASAAARADHYTPGLRPLPKRRLLYSFALLLAVLQAVFVPVTANPAHNRPAGLQRPEESPSRGPCLAGQYLSEGNCKPCREGIDYTSHSNHSLDSCILCTVCKEDKVVETRCNITTNTVCRCKPGTFEDKDSPEICQSCSNCTDGEEELTSCTPRENRKCVSKTAWASWHKLGLWIGLLVPVVLLIGALLVWKTGAWRQWLLCIKRGCERDPESANSVHSSLLDRQTSSTTNDSNHNTEPGKTQKTGKKLLVPVNGNDSADDLKFIFEYCSDIVPFDSWNRLMRQLGLTDNQIQMVKAETLVTREALYQMLLKWRHQTGRSASINHLLDALEAVEERDAMEKIEDYAVKSGRFTYQNAAAQPETGPGGSQCV

SEQ ID NO: 27 - protein, 453 aa, synthetic construct
  REGION 1..453: note = N/A
MEQRGQNAPAASGARKRHGPGPREARGARPGLRVPKTLVLVVAAVLLLVSAESALITQQDLAPQQRVAPQQKRSSPSEGLCPPGHHISEDGRDCISCKYGQDYSTHWNDLLFCLRCTRCDSGEVELSPCTTTRNTVCQCEEGTFREEDSPEMCRKCRTGCPRGMVKVGDCTPWSDIECVHKESGTKHSGEAPAVEETVTSSPGTPASPCSPKSCDKTHTCPPCPAPEAEGAPSVFLFPPKPKDTLMISRTPEVTCVVVDVSHEDPEVKFNWYVDGVEVHNAKTKPREEQYNSTYRVVSVLTVLHQDWLNGKEYKCKVSNKALPAPIEKTISKAKGQPREPQVYTLPPSREEMTKNQVSLTCLVKGFYPSDIAVEWESNGQPENNYKTAPPVLDSDGSFFLYSKLTVDKSRWQQGNVFSCSVMHEALHNHYTQKSLSLSPGKHHHHHHHHEPEA

SEQ ID NO: 28 - protein, 192 aa, synthetic construct
  REGION 1..192: note = N/A
MEQRGQNAPAASGARKRHGPGPREARGARPGPRVPKTLVLVVAAVLLLVSAESALITQQDLAPQQRAAPQQKRSSPSEGLCPPGHHISEDGRDCISCKYGQDYSTHWNDLLFCLRCTRCDSGEVELSPCTTTRNTVCQCEEGTFREEDSPEMCRKCRTGCPRGMVKVGDCTPWSDIECVHKESGHHHHHHHH

SEQ ID NO: 29 - protein, 329 aa, Homo sapiens
STKGPSVFPLAPSSKSTSGGTAALGCLVKDYFPEPVTVSWNSGALTSGVHTFPAVLQSSGLYSLSSVVTVPSSSLGTQTYICNVNHKPSNTKVDKRVEPKSCDKTHTCPPCPAPELLGGPSVFLFPPKPKDTLMISRTPEVTCVVVDVSHEDPEVKFNWYVDGVEVHNAKTKPREEQYNSTYRVVSVLTVLHQDWLNGKEYKCKVSNKALPAPIEKTISKAKGQPREPQVYTLPPSREEMTKNQVSLTCLVKGFYPSDIAVEWESNGQPENNYKTTPPVLDSDGSFFLYSKLTVDKSRWQQGNVFSCSVMHEALHNHYTQKSLSLSPGK

SEQ ID NO: 30 - protein, 329 aa, Homo sapiens
STKGPSVFPLAPSSKSTSGGTAALGCLVKDYFPEPVTVSWNSGALTSGVHTFPAVLQSSGLYSLSSVVTVPSSSLGTQTYICNVNHKPSNTKVDKKVEPKSCDKTHTCPPCPAPELLGGPSVFLFPPKPKDTLMISRTPEVTCVVVDVSHEDPEVKFNWYVDGVEVHNAKTKPREEQYNSTYRVVSVLTVLHQDWLNGKEYKCKVSNKALPAPIEKTISKAKGQPREPQVYTLPPSREEMTKNQVSLTCLVKGFYPSDIAVEWESNGQPENNYKTTPPVLDSDGSFFLYSKLTVDKSRWQQGNVFSCSVMHEALHNHYTQKSLSLSPGK

SEQ ID NO: 31 - protein, 329 aa, Homo sapiens
STKGPSVFPLAPSSKSTSGGTAALGCLVKDYFPEPVTVSWNSGALTSGVHTFPAVLQSSGLYSLSSVVTVPSSSLGTQTYICNVNHKPSNTKVDKPVEPKSCDKTHTCPPCPAPELLGGPSVFLFPPKPKDTLMISRTPEVTCVVVDVSHEDPEVKFNWYVDGVEVHNAKTKPREEQYNSTYRVVSVLTVLHQDWLNGKEYKCKVSNKALPAPIEKTISKAKGQPREPQVYTLPPSRDELTKNQVSLTCLVKGFYPSDIAVEWESNGQPENNYKTTPPVLDSDGSFFLYSKLTVDKSRWQQGNVFSCSVMHEALHNHYTQKSLSLSPGK

SEQ ID NO: 32 - protein, 329 aa, Homo sapiens
STKGPSVFPLAPSSKSTSGGTAALGCLVKDYFPEPVTVSWNSGALTSGVHTFPAVLQSSGLYSLSSVVTVPSSSLGTQTYICNVNHKPSNTKVDKPVEPKSCDKTHTCPPCPAPELLGGPSVFLFPPKPKDTLMISRTPEVTCVVVDVSHEDPEVKFNWYVDGVEVHNAKTKPREEQYNSTYRVVSVLTVLHQDWLNGKEYKCKVSNKALPAPIEKTISKAKGQPREPQVYTLPPSREEMTKNQVSLTCLVKGFYPSDIAVEWESNGQPENNYKTTPPVLDSDGSFFLYSKLTVDKSRWQQGNVFSCSVMHEGLHNHYTQKSLSLSPGK

SEQ ID NO: 33 - protein, 448 aa, synthetic construct
  REGION 1..448: note = N/A
EVQLQQSGAEVVKPGASVKLSCKASGFNIKDTFIHWVKQAPGQGLEWIGRIDPANGNTKYDPKFQGKATITTDTSSNTAYMELSSLRSEDTAVYYCVRGLYTYYFDYWGQGTLVTVSSASTKGPSVFPLAPSSKSTSGGTAALGCLVKDYFPEPVTVSWNSGALTSGVHTFPAVLQSSGLYSLSSVVTVPSSSLGTQTYICNVNHKPSNTKVDKRVEPKSCDKTHTCPPCPAPELLGGPSVFLFPPKPKDTLMISRTPEVTCVVVDVSHEDPEVKFNWYVDGVEVHNAKTKPREEQYNSTYRVVSVLTVLHQDWLNGKEYKCKVSNKALPAPIEKTISKAKGQPREPQVYTLPPSREEMTKNQVSLTCLVKGFYPSDIAVEWESNGQPENNYKTTPPVLDSDGSFFLYSKLTVDKSRWQQGNVFSCSVMHEALHNHYTQKSLSLSPGK

SEQ ID NO: 34 - protein, 448 aa, synthetic construct
  REGION 1..448: note = N/A
EVQLQQSGAEVVKPGASVKLSCKASGFNIKDTFIHWVKQAPGQGLEWIGRIDPANGNTKYDPKFQGKATITTDTSSNTAYMELSSLRSEDTAVYYCVRGLYTYYFDYWGQGTLVTVSSASTKGPSVFPLAPSSKSTSGGTAALGCLVKDYFPEPVTVSWNSGALTSGVHTFPAVLQSSGLYSLSSVVTVPSSSLGTQTYICNVNHKPSNTKVDKRVEPKSCDKTHTCPPCPAPELLGGPSVFLFPPKPKDTLMISRTPEVTCVVVDVSHEDPEVKFNWYVDGVEVHNAKTKPREEQYNSTYRVVSVLTVLHQDWLNGKEYKCKVSNKALPAPIEKTISKAKGQPRKPQVYTLPPSREEMTKNQVSLTCLVKGFYPSDIAVEWESNGQPENNYKTTPPVLDSDGSFFLYSKLTVDKSRWQQGNVFSCSVMHEALHNHYTQKSLSLSPGK

SEQ ID NO: 35 - protein, 448 aa, synthetic construct
  REGION 1..448: note = N/A
EVQLQQSGAEVVKPGASVKLSCKASGFNIKDTFIHWVKQAPGQGLEWIGRIDPANGNTKYDPKFQGKATITTDTSSNTAYMELSSLRSEDTAVYYCVRGLYTYYFDYWGQGTLVTVSSASTKGPSVFPLAPSSKSTSGGTAALGCLVKDYFPEPVTVSWNSGALTSGVHTFPAVLQSSGLYSLSSVVTVPSSSLGTQTYICNVNHKPSNTKVDKRVEPKSCDKTHTCPPCPAPELLGGPSVFLFPPKPKDTLMISRTPEVTCVVVDVSHEDPEVKFNWYVDGVEVHNAKTKPREEQYNSTYRVVSVLTVLHQDWLNGKEYKCKVSNKALPAPIEKTISKAKGQPREPQVYTLPPSREEMTKNQVSLTCLVKGFYPSDIAVEWESNGQPENNYKTTPPVLDSDGSFFLYSKLTVDKSRWQQGNVFSCSVMHGALHNHYTQKSLSLSPGK

SEQ ID NO: 36 - protein, 448 aa, synthetic construct
  REGION 1..448: note = N/A
EVQLQQSGAEVVKPGASVKLSCKASGFNIKDTFIHWVKQAPGQGLEWIGRIDPANTNTKYDPKFQGKATITTDTSSNTAYMELSSLRSEDTAVYYCVRGLYTYYFDYWGQGTLVTVSSASTKGPSVFPLAPSSKSTSGGTAALGCLVKDYFPEPVTVSWNSGALTSGVHTFPAVLQSSGLYSLSSVVTVPSSSLGTQTYICNVNHKPSNTKVDKRVEPKSCDKTHTCPPCPAPELLGGPSVFLFPPKPKDTLMISRTPEVTCVVVDVSHEDPEVKFNWYVDGVEVHNAKTKPREEQYNSTYRVVSVLTVLHQDWLNGKEYKCKVSNKALPAPIEKTISKAKGQPREPQVYTLPPSREEMTKNQVSLTCLVKGFYPSDIAVEWESNGQPENNYKTTPPVLDSDGSFFLYSKLTVDKSRWQQGNVFSCSVMHEALHNHYTQKSLSLSPGK

SEQ ID NO: 37 - protein, 448 aa, synthetic construct
  REGION 1..448: note = N/A
EVQLQQSGAEVVKPGASVKLSCKASGFNIKDTFIHWVKQAPGQGLEWIGRIDPANTNTKYDPKFQGKATITTDTSSNTAYMELSSLRSEDTAVYYCVRGLYTYYFDYWGQGTLVTVSSASTKGPSVFPLAPSSKSTSGGTAALGCLVKDYFPEPVTVSWNSGALTSGVHTFPAVLQSSGLYSLSSVVTVPSSSLGTQTYICNVNHKPSNTKVDKRVEPKSCDKTHTCPPCPAPELLGGPSVFLFPPKPKDTLMISRTPEVTCVVVDVSHEDPEVKFNWYVDGVEVHNAKTKPREEQYNSTYRVVSVLTVLHQDWLNGKEYKCKVSNKALPAPIEKTISKAKGQPRKPQVYTLPPSREEMTKNQVSLTCLVKGFYPSDIAVEWESNGQPENNYKTTPPVLDSDGSFFLYSKLTVDKSRWQQGNVFSCSVMHEALHNHYTQKSLSLSPGK

SEQ ID NO: 38 - protein, 448 aa, synthetic construct
  REGION 1..448: note = N/A
EVQLQQSGAEVVKPGASVKLSCKASGFNIKDTFIHWVKQAPGQGLEWIGRIDPANTNTKYDPKFQGKATITTDTSSNTAYMELSSLRSEDTAVYYCVRGLYTYYFDYWGQGTLVTVSSASTKGPSVFPLAPSSKSTSGGTAALGCLVKDYFPEPVTVSWNSGALTSGVHTFPAVLQSSGLYSLSSVVTVPSSSLGTQTYICNVNHKPSNTKVDKRVEPKSCDKTHTCPPCPAPELLGGPSVFLFPPKPKDTLMISRTPEVTCVVVDVSHEDPEVKFNWYVDGVEVHNAKTKPREEQYNSTYRVVSVLTVLHQDWLNGKEYKCKVSNKALPAPIEKTISKAKGQPREPQVYTLPPSREEMTKNQVSLTCLVKGFYPSDIAVEWESNGQPENNYKTTPPVLDSDGSFFLYSKLTVDKSRWQQGNVFSCSVMHGALHNHYTQKSLSLSPGK

SEQ ID NO: 39 - protein, 214 aa, synthetic construct
  REGION 1..214: note = N/A
EIVMTQSPATLSVSPGERATLSCRASQSISNNLHWYQQKPGQAPRLLIKFASQSITGIPARFSGSGSGTEFTLTISSLQSEDFAVYYCQQGNSWPYTFGQGTKLEIKRTVAAPSVFIFPPSDEQLKSGTASVVCLLNNFYPREAKVQWKVDNALQSGNSQESVTEQDSKDSTYSLSSTLTLSKADYEKHKVYACEVTHQGLSSPVTKSFNRGEC

SEQ ID NO: 40 - protein, 448 aa, synthetic construct
  REGION 1..448: note = N/A
QVQLVQSGAEVKKPGASVKVSCKASGFNIKDTHMHWVRQAPGQRLEWIGRIDPANGNTEYDQKFQGRVTITVDTSASTAYMELSSLRSEDTAVYYCARWGTNVYFAYWGQGTLVTVSSASTKGPSVFPLAPSSKSTSGGTAALGCLVKDYFPEPVTVSWNSGALTSGVHTFPAVLQSSGLYSLSSVVTVPSSSLGTQTYICNVNHKPSNTKVDKRVEPKSCDKTHTCPPCPAPELLGGPSVFLFPPKPKDTLMISRTPEVTCVVVDVSHEDPEVKFNWYVDGVEVHNAKTKPREEQYNSTYRVVSVLTVLHQDWLNGKEYKCKVSNKALPAPIEKTISKAKGQPREPQVYTLPPSREEMTKNQVSLTCLVKGFYPSDIAVEWESNGQPENNYKTTPPVLDSDGSFFLYSKLTVDKSRWQQGNVFSCSVMHEALHNHYTQKSLSLSPGK

SEQ ID NO: 41 - protein, 448 aa, synthetic construct
  REGION 1..448: note = N/A
QVQLVQSGAEVKKPGASVKVSCKASGFNIKDTHMHWVRQAPGQRLEWIGRIDPANGNTEYDQKFQGRVTITVDTSASTAYMELSSLRSEDTAVYYCARWGTNVYFAYWGQGTLVTVSSASTKGPSVFPLAPSSKSTSGGTAALGCLVKDYFPEPVTVSWNSGALTSGVHTFPAVLQSSGLYSLSSVVTVPSSSLGTQTYICNVNHKPSNTKVDKRVEPKSCDKTHTCPPCPAPELLGGPSVFLFPPKPKDTLMISRTPEVTCVVVDVSHEDPEVKFNWYVDGVEVHNAKTKPREEQYNSTYRVVSVLTVLHQDWLNGKEYKCKVSNKALPAPIEKTISKAKGQPRKPQVYTLPPSREEMTKNQVSLTCLVKGFYPSDIAVEWESNGQPENNYKTTPPVLDSDGSFFLYSKLTVDKSRWQQGNVFSCSVMHEALHNHYTQKSLSLSPGK

SEQ ID NO: 42 - protein, 448 aa, synthetic construct
  REGION 1..448: note = N/A
QVQLVQSGAEVKKPGASVKVSCKASGFNIKDTHMHWVRQAPGQRLEWIGRIDPANGNTEYDQKFQGRVTITVDTSASTAYMELSSLRSEDTAVYYCARWGTNVYFAYWGQGTLVTVSSASTKGPSVFPLAPSSKSTSGGTAALGCLVKDYFPEPVTVSWNSGALTSGVHTFPAVLQSSGLYSLSSVVTVPSSSLGTQTYICNVNHKPSNTKVDKRVEPKSCDKTHTCPPCPAPELLGGPSVFLFPPKPKDTLMISRTPEVTCVVVDVSHEDPEVKFNWYVDGVEVHNAKTKPREEQYNSTYRVVSVLTVLHQDWLNGKEYKCKVSNKALPAPIEKTISKAKGQPREPQVYTLPPSREEMTKNQVSLTCLVKGFYPSDIAVEWESNGQPENNYKTTPPVLDSDGSFFLYSKLTVDKSRWQQGNVFSCSVMHGALHNHYTQKSLSLSPGK

SEQ ID NO: 43 - protein, 213 aa, synthetic construct
  REGION 1..213: note = N/A
DIQLTQSPSSLSASVGDRVTITCSASSSVSYMYWYQQKPGKAPKPWIYRTSNLASGVPSRFSGSGSGTDFTLTISSLQPEDFATYYCQQYHSYPPTFGGGTKVEIKRTVAAPSVFIFPPSDEQLKSGTASVVCLLNNFYPREAKVQWKVDNALQSGNSQESVTEQDSKDSTYSLSSTLTLSKADYEKHKVYACEVTHQGLSSPVTKSFNRGEC

SEQ ID NO: 44 - protein, 440 aa, Homo sapiens
MEQRGQNAPAASGARKRHGPGPREARGARPGPRVPKTLVLVVAAVLLLVSAESALITQQDLAPQQRAAPQQKRSSPSEGLCPPGHHISEDGRDCISCKYGQDYSTHWNDLLFCLRCTRCDSGEVELSPCTTTRNTVCQCEEGTFREEDSPEMCRKCRTGCPRGMVKVGDCTPWSDIECVHKESGTKHSGEVPAVEETVTSSPGTPASPCSLSGIIIGVTVAAVVLIVAVFVCKSLLWKKVLPYLKGICSGGGGDPERVDRSSQRPGAEDNVLNEIVSILQPTQVPEQEMEVQEPAEPTGVNMLSPGESEHLLEPAEAERSQRRRLLVPANEGDPTETLRQCFDDFADLVPFDSWEPLMRKLGLMDNEIKVAKAEAAGHRDTLYTMLIKWVNKTGRDASVHTLLDALETLGERLANQKIEDHLLSSGKFMYLEGNADSAMS

SEQ ID NO: 45 - protein, 440 aa, Homo sapiens [sequence omitted]

SEQ ID NO: 46 - protein, 440 aa, Homo sapiens
MEQRGQNAPAASGARKRHGPGPREARGARPGPRVPKTLVLVVAAVLLLVSAESALITQQDLAPQQRAAPQQKRSSPSEGLCPPGHHISEDGRDCISCKYGQDYSTHWNDLLFCLRCTRCDSGEVELSPCTTTRNTVCQCEEGTFREEDSPEMCRKCRTGCPRGMVKVGDCTPWSDIECVHKESGTKHSGEVPAVEETVTSSPGTPASPCSLSGIIIGVTVAAVVLIVAVFVCKSLLWKKVLPYLKGICSGGGGDPERVDRSSQRPGAEDNVLNEIVSILQPTQVPEQEMEVQEPAEPTGVNMLSPGESEHLLEPAEAERSQRRRLLVPANEGDPTETLRQCFDDFADLVPFDSWEPLMRKLGLMDNEIKVAKAEAAGHRDTLYTMLIKWVNKTGRDASVHTLLDALETLGERLAKQKIEDHLLSSGKFMYLEGNADSAMS

SEQ ID NO: 47 - protein, 411 aa, Homo sapiens
MEQRGQNAPAASGARKRHGPGPREARGARPGPRVPKTLVLVVAAVLLLVSAESALITQQDLAPQQRAAPQQKRSSPSEGLCPPGHHISEDGRDCISCKYGQDYSTHWNDLLFCLRCTRCDSGEVELSPCTTTRNTVCQCEEGTFREEDSPEMCRKCRTGCPRGMVKVGDCTPWSDIECVHKESGIIIGVTVAAVVLIVAVFVCKSLLWKKVLPYLKGICSGGGGDPERVDRSSQRPGAEDNVLNEIVSILQPTQVPEQEMEVQEPAEPTGVNMLSPGESEHLLEPAEAERSQRRRLLVPANEGDPTETLRQCFDDFADLVPFDSWEPLMRKLGLMDNEIKVAKAEAAGHRDTLYTMLIKWVNKTGRDASVHTLLDALETLGERLANQKIEDHLLSSGKFMYLEGNADSAMS

SEQ ID NO: 48 - protein, 445 aa, Macaca fascicularis
MGQLRQSAPAASGARKGRGPGPREARGARPGLRVLKTLVLVVAAARVLLSVSADCAPITRQSLDPQRRAAPQQKRSSPTEGLCPPGHHISEDSRECISCKYGQDYSTHWNDFLFCLRCTKCDSGEVEVNSCTTTRNTVCQCEEGTFREEDSPEICRKCRTGCPRGMVKVKDCTPWSDIECVHKESGTKHTGEVPAVEKTVTTSPGTPASPCSLSGIIIGVIVLVVIVVVAVIVWKTSLWKKVLPYLKGVCSGGGGDPERVDSSSHSPQRPGAEDNALNEIVSIVQPSQVPEQEMEVQEPAEQTDVNTLSPGESEHLLEPAKAEGPQRRGQLVPVNENDPTETLRQCFDDFAAIVPFDAWEPLVRQLGLTNNEIKVAKAEAASSRDTLYVMLIKWVNKTGRAASVNTLLDALETLEERLAKQKIQDRLLSSGKFMYLEDNADSATS

SEQ ID NO: 49 - protein, 445 aa, Macaca fascicularis
MGQLRQSAPAASGARKGRGPGPREARGARPGLRVLKTLVLVVAAARVLLSVSADCAPITRQSLDPQRRAAPQQKRSSPTEGLCPPGHHISEDSRECISCKYGQDYSTHWNDFLFCLRCTKCDSGEVEVNSCTTTRNTVCQCEEGTFREEDSPEICRKCRTGCPRGMVKVKDCTPWSDIECVHKESGTKHTGEVPAVEKTVTTSPGTPASPCSLSGIIIGVIVLVVIVVVAVIVWKTSLWKKVLPYLKGVCSGGGGDPERVDSSSHSPQRPGAEDNALNEIVSIVQPSQVPEQEMEVQEPAEQTDVNTLSPGESEHLLEPAKAEGPQRRGQLVPVNENDPTETLRQCFDDFAAIVPFDAWEPLVRQLGLTNNEIKVAKAEAASSRDTLYVMLIKWVNKTGRAASVNTLLDALETLEERLANQKIQDRLLSSGKFMYLEDNADSATS

SEQ ID NO: 50 - protein, 416 aa, Macaca fascicularis
MGQLRQSAPAASGARKGRGPGPREARGARPGLRVLKTLVLVVAAARVLLSVSADCAPITRQSLDPQRRAAPQQKRSSPTEGLCPPGHHISEDSRECISCKYGQDYSTHWNDFLFCLRCTKCDSGEVEVNSCTTTRNTVCQCEEGTFREEDSPEICRKCRTGCPRGMVKVKDCTPWSDIECVHKESGIIIGVIVLVVIVVVAVIVWKTSLWKKVLPYLKGVCSGGGGDPERVDSSSHSPQRPGAEDNALNEIVSIVQPSQVPEQEMEVQEPAEQTDVNTLSPGESEHLLEPAKAEGPQRRGQLVPVNENDPTETLRQCFDDFAAIVPFDAWEPLVRQLGLTNNEIKVAKAEAASSRDTLYVMLIKWVNKTGRAASVNTLLDALETLEERLANQKIQDRLLSSGKFMYLEDNADSATS

SEQ ID NO: 51 - protein, 8 aa, synthetic construct
  REGION 1..8: note = N/A
GFTFSSYV

SEQ ID NO: 52 - protein, 8 aa, synthetic construct
  REGION 1..8: note = N/A
ISSGGSYT

SEQ ID NO: 53 - protein, 12 aa, synthetic construct
  REGION 1..12: note = N/A
ARRGDSMITTDY

SEQ ID NO: 54 - protein, 6 aa, synthetic construct
  REGION 1..6: note = N/A
QDVGTA

SEQ ID NO: 55 - protein, 8 aa, synthetic construct
  REGION 1..8: note = N/A
QQYSSYRT

SEQ ID NO: 56 - protein, 449 aa, synthetic construct
  REGION 1..449: note = N/A
EVMLVESGGGLVKPGGSLKLSCAASGFTFSSYVMSWVRQTPEKRLEWVATISSGGSYTYYPDSVKGRFTISRDNAKNTLYLQMSSLRSEDTAMYYCARRGDSMITTDYWGQGTTLTVSSASTKGPSVFPLAPSSKSTSGGTAALGCLVKDYFPEPVTVSWNSGALTSGVHTFPAVLQSSGLYSLSSVVTVPSSSLGTQTYICNVNHKPSNTKVDKRVEPKSCDKTHTCPPCPAPELLGGPSVFLFPPKPKDTLMISRTPEVTCVVVDVSHEDPEVKFNWYVDGVEVHNAKTKPREEQYNSTYRVVSVLTVLHQDWLNGKEYKCKVSNKALPAPIEKTISKAKGQPREPQVYTLPPSREEMTKNQVSLTCLVKGFYPSDIAVEWESNGQPENNYKTTPPVLDSDGSFFLYSKLTVDKSRWQQGNVFSCSVMHEALHNHYTQKSLSLSPGK

SEQ ID NO: 57 - protein, 213 aa, synthetic construct
  REGION 1..213: note = N/A
DIVMTQSHKFMSTSVGDRVSITCKASQDVGTAVAWYQQKPGQSPKLLIYWASTRHTGVPDRFTGSGSGTDFTLTISNVQSEDLADYFCQQYSSYRTFGGGTKLEIKRTVAAPSVFIFPPSDEQLKSGTASVVCLLNNFYPREAKVQWKVDNALQSGNSQESVTEQDSKDSTYSLSSTLTLSKADYEKHKVYACEVTHQGLSSPVTKSFNRGEC

SEQ ID NO: 58 - protein, 329 aa, synthetic construct
  REGION 1..329: note = N/A
STKGPSVFPLAPSSKSTSGGTAALGCLVKDYFPEPVTVSWNSGALTSGVHTFPAVLQSSGLYSLSSVVTVPSSSLGTQTYICNVNHKPSNTKVDKRVEPKSCDKTHTCPPCPAPELLGGPSVFLFPPKPKDTLMISRTPEVTCVVVDVSHEDPEVKFNWYVDGVEVHNAKTKPREEQYNSTYRVVSVLTVLHQDWLNGKEYKCKVSNKALPAPIEKTISKAKGQPREPQVYTLPPSREEMTKNQVSLTCLVKGFYPSDIAVEWESNGQPENNYKTTPPVLDSDGSFFLYSKLTVDKSRWQQGNVFSCSVMHGALHNHYTQKSLSLSPGK

SEQ ID NO: 59 - protein, 329 aa, synthetic construct
  REGION 1..329: note = N/A
STKGPSVFPLAPSSKSTSGGTAALGCLVKDYFPEPVTVSWNSGALTSGVHTFPAVLQSSGLYSLSSVVTVPSSSLGTQTYICNVNHKPSNTKVDKRVEPKSCDKTHTCPPCPAPELLGGPSVFLFPPKPKDTLMISRTPEVTCVVVDVSHEDPEVKFNWYVDGVEVHNAKTKPREEQYNSTYRVVSVLTVLHQDWLNGKEYKCKVSNKALPAPIEKTISKAKGQPRKPQVYTLPPSREEMTKNQVSLTCLVKGFYPSDIAVEWESNGQPENNYKTTPPVLDSDGSFFLYSKLTVDKSRWQQGNVFSCSVMHEALHNHYTQKSLSLSPGK

SEQ ID NO: 60 - protein, 329 aa, synthetic construct
  REGION 1..329: note = N/A
STKGPSVFPLAPSSKSTSGGTAALGCLVKDYFPEPVTVSWNSGALTSGVHTFPAVLQSSGLYSLSSVVTVPSSSLGTQTYICNVNHKPSNTKVDKRVEPKSCDKTHTCPPCPAPELLGGPSVFLFPPKPKDTLMISRTPEVTCVVVDVSHEDPEVKFNWYVDGVEVHNAKTKPREEQYNSTYRVVSVLTVLHQDWLNGKEYKCKVSNKALPAPIEKTISKAKGQPREPQVYTLPPSREEMTKNQVSLTCLVKGFYPSDIAVEWESNGQPENNYKTTPPVLDSDGSFFLYSKLTVDKSRWQQGNVFSCSVMHEALHNHYTQKYLSLSPGK

SEQ ID NO: 61 - protein, 329 aa, synthetic construct
  REGION 1..329: note = N/A
STKGPSVFPLAPSSKSTSGGTAALGCLVKDYFPEPVTVSWNSGALTSGVHTFPAVLQSSGLYSLSSVVTVPSSSLGTQTYICNVNHKPSNTKVDKRVEPKSCDKTHTCPPCPAPELLGGPSVFLFPPKPKDTLMISRTPEVTCVVVDVSHEDPEVKFNWYVDGVEVHNAKTKPREEQYNSTYRVVSVLTVLHQDWLNGKEYKCKVSNKALPAPIEKTISKAKGQPREPQVYTLPPSREEMTKNQVSLTCLVKGFYPSDIAVEWESNGQPENNYKTTPPVLDSDGSFFLYSKLTVDKSRWQQGNVFSCSVMHGALHNHYTQESLSLSPGK

SEQ ID NO: 62 - protein, 329 aa, synthetic construct
  REGION 1..329: note = N/A
STKGPSVFPLAPSSKSTSGGTAALGCLVKDYFPEPVTVSWNSGALTSGVHTFPAVLQSSGLYSLSSVVTVPSSSLGTQTYICNVNHKPSNTKVDKRVEPKSCDKTHTCPPCPAPELLGGPSVFLFPPKPKDTLMISRTPEVTCVVVDVSHEDPEVKFNWYVDGVEVHNAKTKPREEQYNSTYRVVSVLTVLHQDWLNGKEYKCKVSNKALPAPIEKTISKAKGQPREPQVYTLPPSREEMTKNQVSLTCLVKGFYPSDIAVEWESNGQPENNYKTTPPVLDSDGSFFLYSKLTVDKSRWQQGNVFSCSVMHGALHNHYTQKKLSLSPGK

SEQ ID NO: 63 - protein, 329 aa, synthetic construct
  REGION 1..329: note = N/A
STKGPSVFPLAPSSKSTSGGTAALGCLVKDYFPEPVTVSWNSGALTSGVHTFPAVLQSSGLYSLSSVVTVPSSSLGTQTYICNVNHKPSNTKVDKRVEPKSCDKTHTCPPCPAPELLGGPSVFLFPPKPKDTLMISRTPEVTCVVVDVSHEDPEVKFNWYVDGVEVHNAKTKPREEQYNSTYRVVSVLTVLHQDWLNGKEYKCKVSNKALPAPIEKTISKAKGQPREPQVYTLPPSREEMTKNQVSLTCLVKGFYPSDIAVEWESNGQPENNYKTTPPVLDSDGSFFLYSRLTVDKSRWQQGNVFSCSVMHEALHNHYTQKSLSLSPGK

SEQ ID NO: 64 - protein, 329 aa, synthetic construct
  REGION 1..329: note = N/A
STKGPSVFPLAPSSKSTSGGTAALGCLVKDYFPEPVTVSWNSGALTSGVHTFPAVLQSSGLYSLSSVVTVPSSSLGTQTYICNVNHKPSNTKVDKRVEPKSCDKTHTCPPCPAPELLGGPSVFLFPPKPKDTLMISRTPEVTCVVVDVSHEDPEVKFNWYVDGVEVHNAKTKPREEQYNSTYRVVSVLTVLHQDWLNGKEYKCKVSNKALPAPIEKTISKAKGQPRKPQVYTLPPSREEMTKNQVSLTCLVKGFYPSDIAVEWESNGQPENNYKTTPPVLDSDGSFFLYSRLTVDKSRWQQGNVFSCSVMHEALHNHYTQKSLSLSPGK

SEQ ID NO: 65 - protein, 329 aa, synthetic construct
  REGION 1..329: note = N/A
STKGPSVFPLAPSSKSTSGGTAALGCLVKDYFPEPVTVSWNSGALTSGVHTFPAVLQSSGLYSLSSVVTVPSSSLGTQTYICNVNHKPSNTKVDKRVEPKSCDKTHTCPPCPAPELLGGPSVFLFPPKPKDTLMISRTPEVTCVVVDVSHEDPEVKFNWYVDGVEVHNAKTKPREEQYNSTYRVVSVLTVLHQDWLNGKEYKCKVSNKALPAPIEKTISKAKGQPREPQVYTLPPSREEMTKNQVSLTCLVKGFYPSDIAVEWESNGQPENNYKTTPPVLDSDGSFFLYSRLTVDKSRWQQGNVFSCSVMHGALHNHYTQKSLSLSPGK

SEQ ID NO: 66 - protein, 329 aa, synthetic construct
  REGION 1..329: note = N/A
STKGPSVFPLAPSSKSTSGGTAALGCLVKDYFPEPVTVSWNSGALTSGVHTFPAVLQSSGLYSLSSVVTVPSSSLGTQTYICNVNHKPSNTKVDKRVEPKSCDKTHTCPPCPAPELLGGPSVFLFPPKPKDTLMISRTPEVTCVVVDVSHEDPEVKFNWYVDGVEVHNAKTKPREEQYNSTYRVVSVLTVLHQDWLNGKEYKCKVSNKALPAPIEKTISKAKGQPREPQVYTLPPSREEMTKNQVSLTCLVKGFYPSDIAVEWESNGQPENNYKTTPPVLDSDGSFLLYSKLTVDKSRWQQGNVFSCSVMHEALHNHYTQKSLSLSPGK

SEQ ID NO: 67 - protein, 329 aa, synthetic construct
  REGION 1..329: note = N/A
STKGPSVFPLAPSSKSTSGGTAALGCLVKDYFPEPVTVSWNSGALTSGVHTFPAVLQSSGLYSLSSVVTVPSSSLGTQTYICNVNHKPSNTKVDKRVEPKSCDKTHTCPPCPAPELLGGPSVFLFPPKPKDTLMISRTPEVTCVVVDVSHEDPEVKFNWYVDGVEVHNAKTKPREEQYNSTYRVVSVLTVLHQDWLNGKEYKCKVSNKALPAPIEKTISKAKGQPRKPQVYTLPPSREEMTKNQVSLTCLVKGFYPSDIAVEWESNGQPENNYKTTPPVLDSDGSFLLYSKLTVDKSRWQQGNVFSCSVMHEALHNHYTQKSLSLSPGK

SEQ ID NO: 68 - protein, 329 aa, synthetic construct
  REGION 1..329: note = N/A
STKGPSVFPLAPSSKSTSGGTAALGCLVKDYFPEPVTVSWNSGALTSGVHTFPAVLQSSGLYSLSSVVTVPSSSLGTQTYICNVNHKPSNTKVDKRVEPKSCDKTHTCPPCPAPELLGGPSVFLFPPKPKDTLMISRTPEVTCVVVDVSHEDPEVKFNWYVDGVEVHNAKTKPREEQYNSTYRVVSVLTVLHQDWLNGKEYKCKVSNKALPAPIEKTISKAKGQPREPQVYTLPPSREEMTKNQVSLTCLVKGFYPSDIAVEWESNGQPENNYKTTPPVLDSDGSFLLYSKLTVDKSRWQQGNVFSCSVMHGALHNHYTQKSLSLSPGK